European Patent Specification EP 4 042 167 B1, published April 9, 2025. Title: Compositions and Methods for an IL-17 Target Engagement Assay with Large Molecule Modulators. Applicant: Janssen Biotech, Inc. The sequence listing filed with the application follows.

SEQUENCE LISTING (23 sequences)

SEQ ID NO: 1 - protein, 12 aa, Artificial Sequence
  LCDR1 of mAb4538 and mAb732
RASQNVWAFYLA

SEQ ID NO: 2 - protein, 7 aa, Artificial Sequence
  LCDR2 of mAb4538 and mAb732
GASNRAT

SEQ ID NO: 3 - protein, 10 aa, Artificial Sequence
  LCDR3 of mAb4538
QQYRSTLSLT

SEQ ID NO: 4 - protein, 7 aa, Artificial Sequence
  HCDR1 of mAb4538 and mAb732
SSSAAWG

SEQ ID NO: 5 - protein, 18 aa, Artificial Sequence
  HCDR2 of mAb4538 and mAb732
RISYRSKWYNDYAVSVKS

SEQ ID NO: 6 - protein, 12 aa, Artificial Sequence
  HCDR3 of mAb4538 and mAb732
EVDSMYYSYFDI

SEQ ID NO: 7 - protein, 109 aa, Artificial Sequence
  VL of mAb4538
EIVLTQSPATLSLSPGERATLSCRASQNVWAFYLAWYQQKPGQAPRLLIYGASNRATGIPARFSGSGSGTDFTLTISSLEPEDFAVYYCQQYRSTLSLTFGQGTKVEIK

SEQ ID NO: 8 - protein, 124 aa, Artificial Sequence
  VH of mAb4538 and mAb732
QVQLQQSGPGLVKPSQTLSLTCAISGDSVSSSSAAWGWIRQSPSRGLEWLGRISYRSKWYNDYAVSVKSRITINPDTSKNQFSLQLNSVTPEDTAVYYCAREVDSMYYSYFDIWGQGTLVTVSS

SEQ ID NO: 9 - protein, 215 aa, Artificial Sequence
  LC of mAb4538
EIVLTQSPATLSLSPGERATLSCRASQNVWAFYLAWYQQKPGQAPRLLIYGASNRATGIPARFSGSGSGTDFTLTISSLEPEDFAVYYCQQYRSTLSLTFGQGTKVEIKGQPKAAPSVTLFPPSSEELQANKATLVCLISDFYPGAVTVAWKADSSPVKAGVETTTPSKQSNNKYAASSYLSLTPEQWKSHRSYSCQVTHEGSTVEKTVAPTECS

SEQ ID NO: 10 - protein, 454 aa, Artificial Sequence
  HC of mAb4538 and mAb732
QVQLQQSGPGLVKPSQTLSLTCAISGDSVSSSSAAWGWIRQSPSRGLEWLGRISYRSKWYNDYAVSVKSRITINPDTSKNQFSLQLNSVTPEDTAVYYCAREVDSMYYSYFDIWGQGTLVTVSSASTKGPSVFPLAPSSKSTSGGTAALGCLVKDYFPEPVTVSWNSGALTSGVHTFPAVLQSSGLYSLSSVVTVPSSSLGTQTYICNVNHKPSNTKVDKKVEPKSCDKTHTCPPCPAPELLGGPSVFLFPPKPKDTLMISRTPEVTCVVVDVSHEDPEVKFNWYVDGVEVHNAKTKPREEQYNSTYRVVSVLTVLHQDWLNGKEYKCKVSNKALPAPIEKTISKAKGQPREPQVYTLPPSRDELTKNQVSLTCLVKGFYPSDIAVEWESNGQPENNYKTTPPVLDSDGSFFLYSKLTVDKSRWQQGNVFSCSVMHEALHNHYTQKSLSLSPGK

SEQ ID NO: 11 - protein, 10 aa, Artificial Sequence
  LCDR3 of mAb732
TQYYSSPSLT

SEQ ID NO: 12 - protein, 109 aa, Artificial Sequence
  VL of mAb732
EIVLTQSPATLSLSPGERATLSCRASQNVWAFYLAWYQQKPGQAPRLLIYGASNRATGIPARFSGSGSGTDFTLTISSLEPEDFAVYYCTQYYSSPSLTFGQGTKVEIK

SEQ ID NO: 13 - protein, 11 aa, Artificial Sequence
  LCDR1 of mAb7024
RASQGISNWLN

SEQ ID NO: 14 - protein, 7 aa, Artificial Sequence
  LCDR2 of mAb7024
AASSLQS

SEQ ID NO: 15 - protein, 8 aa, Artificial Sequence
  LCDR3 of mAb7024
QQYSDDPT

SEQ ID NO: 16 - protein, 5 aa, Artificial Sequence
  HCDR1 of mAb7024
SYAIS

SEQ ID NO: 17 - protein, 17 aa, Artificial Sequence
  HCDR2 of mAb7024
SIIPWFGTTNYAQKFQG

SEQ ID NO: 18 - protein, 8 aa, Artificial Sequence
  HCDR3 of mAb7024
DSEYYFDH

SEQ ID NO: 19 - protein, 106 aa, Artificial Sequence
  VL of mAb7024
DIQMTQSPSSVSASVGDRVTITCRASQGISNWLNWYQQKPGKAPKLLIYAASSLQSGVPSRFSGSGSGTDFTLTISSLQPEDFATYYCQQYSDDPTFGQGTKVEIK

SEQ ID NO: 20 - protein, 117 aa, Artificial Sequence
  VH of mAb7024
QVQLVQSGAEVKKPGSSVKVSCKASGGTFSSYAISWVRQAPGQGLEWMGSIIPWFGTTNYAQKFQGRVTITADESTSTAYMELSSLRSEDTAVYYCARDSEYYFDHWGQGTLVTVSS

SEQ ID NO: 21 - protein, 212 aa, Artificial Sequence
  LC of mAb7024
DIQMTQSPSSVSASVGDRVTITCRASQGISNWLNWYQQKPGKAPKLLIYAASSLQSGVPSRFSGSGSGTDFTLTISSLQPEDFATYYCQQYSDDPTFGQGTKVEIKGQPKAAPSVTLFPPSSEELQANKATLVCLISDFYPGAVTVAWKADSSPVKAGVETTTPSKQSNNKYAASSYLSLTPEQWKSHRSYSCQVTHEGSTVEKTVAPTECS

SEQ ID NO: 22 - protein, 215 aa, Artificial Sequence
  LC of mAb732
EIVLTQSPATLSLSPGERATLSCRASQNVWAFYLAWYQQKPGQAPRLLIYGASNRATGIPARFSGSGSGTDFTLTISSLEPEDFAVYYCTQYYSSPSLTFGQGTKVEIKGQPKAAPSVTLFPPSSEELQANKATLVCLISDFYPGAVTVAWKADSSPVKAGVETTTPSKQSNNKYAASSYLSLTPEQWKSHRSYSCQVTHEGSTVEKTVAPTECS

SEQ ID NO: 23 - protein, 447 aa, Artificial Sequence
  HC of mAb7024
QVQLVQSGAEVKKPGSSVKVSCKASGGTFSSYAISWVRQAPGQGLEWMGSIIPWFGTTNYAQKFQGRVTITADESTSTAYMELSSLRSEDTAVYYCARDSEYYFDHWGQGTLVTVSSASTKGPSVFPLAPSSKSTSGGTAALGCLVKDYFPEPVTVSWNSGALTSGVHTFPAVLQSSGLYSLSSVVTVPSSSLGTQTYICNVNHKPSNTKVDKKVEPKSCDKTHTCPPCPAPELLGGPSVFLFPPKPKDTLMISRTPEVTCVVVDVSHEDPEVKFNWYVDGVEVHNAKTKPREEQYNSTYRVVSVLTVLHQDWLNGKEYKCKVSNKALPAPIEKTISKAKGQPREPQVYTLPPSRDELTKNQVSLTCLVKGFYPSDIAVEWESNGQPENNYKTTPPVLDSDGSFFLYSKLTVDKSRWQQGNVFSCSVMHEALHNHYTQKSLSLSPGK